European Patent Specification EP 3 737 423 B1, published September 18, 2024. Title: COMPOSITIONS AND METHODS FOR TREATING RETINAL DISORDERS. Applicant: UCL BUSINESS PLC. The sequence listing filed with the application follows.

SEQUENCE LISTING (17 sequences)

SEQ ID NO: 1 - DNA, 1253 bp, Artificial Sequence
  1.2 kb fragment of the M/L opsin Locus Control Region (LCR)
taggaatagaagggtgggtgcaggaggctgaggggtggggaaagggcatgggtgtttcatgaggacagagcttccgtttcatgcaatgaaaagagtttggagacggatggtggtgactggactatacacttacacacggtagcgatggtacactttgtattatgtatattttaccacgatctttttaaagtgtcaaaggcaaatggccaaatggttccttgtcctatagctgtagcagccatcggctgttagtgacaaagcccctgagtcaagatgacagcagcccccataactcctaatcggctctcccgcgtggagtcatttaggagtagtcgcattagagacaagtccaacatctaatcttccaccctggccagggccccagctggcagcgagggtgggagactccgggcagagcagagggcgctgacattggggcccggcctggcttgggtccctctggcctttccccaggggccctctttccttggggctttcttgggccgccactgctcccgctcctctccccccatcccaccccctcaccccctcgttcttcatatccttctctagtgctccctccactttcatccacccttctgcaagagtgtgggaccacaaatgagttttcacctggcctggggacacacgtgcccccacaggtgctgagtgactttctaggacagtaatctgctttaggctaaaatgggacttgatcttctgttagccctaatcatcaattagcagagccggtgaaggtgcagaacctaccgcctttccaggcctcctcccacctctgccacctccactctccttcctgggatgtgggggctggcacacgtgtggcccagggcattggtgggattgcactgagctgggtcattagcgtaatcctggacaagggcagacagggcgagcggagggccagctccggggctcaggcaaggctgggggcttcccccagacaccccactcctcctctgctggacccccacttcatagggcacttcgtgttctcaaagggcttccaaatagcatggtggccttggatgcccagggaagcctcagagttgcttatctccctctagacagaaggggaatctcggtcaagagggagaggtcgccctgttcaaggccacccagccagctcatggcggtaatgggacaaggctggccagccatcccaccctcagaagggacccggtggggcaggtgatctcagaggaggctcacttctgggtctcacattcttg

SEQ ID NO: 2 - DNA, 1970 bp, Artificial Sequence
  2.0 kb M opsin promoter fragment, with no M8 sequence
taaaaagcaagtcttgccagggcagtggtgtgcacctgtggtcccagctactcaggatgctgaggcaggaggattacttgtgcccagcaagtagaggctgcagtgacctgtgactgtgctactgccctccaacctgggtgacagagtgagaccttgtctcaaaaaaaaaagagcggggggggggggccgggccgggcgtggtggctcacagctgtaatcccagcactttgggaagccaaggcgggtggatcacttgaggtcaggagtttgagaccatcatggtcaacactgcgaaacactgtccctactaaaaatacaaaaattagccgggcatggtggcacacacctgtaatcccagctactggggaggctgaggcaggagaattgcttgagccggggagacggaggttgcagtgagccgagactgcgccactgcactccagcctgactgacaagagtgagattgtctcaaaaaaaaaaaaaaagtaatcactagaaaagaagctacatatgtacataacatccaaataaccaagaggagaaaaaaatgggacttgattaatcaaaacaaaaacaaaaaagaaagaaagaaagggggagaaaataaaacaagggctgggtgtgctggctcatgcctgtaatcccagcactttggaagccaaggtgggtggatctcttgagctcaggaggtcaagaccagcctgggcaacatggcgaaaccccgtctctattaaaaaaaaaattaatacaacaattatcctggagtggtggtgcacacctgtagtcccagctacccaggacgctgagacgggaggatcgcttgatcccggggatgtcgaggctgccgtgatcgcaccactgccctccagccagggtggcagactgagaccccatctcaaaaaataaataaataaaagcaaacaagaaaaaaaaaggcttgaaacatatctgatagataaagggctaatcaacacaatatataaagaactgcaaatcagtaaactaagagcaaataacccaatataaagacattaaagggtagccacggacatctcagacgacgaaaaacaaaagacagtaaacgtataataaaacatgtaattgcaaggtgatccgggaatagtaagcgaaaagcaacaattaaatactattttctcatccaccagaacgccaaaaattaaaaagcctaacaatgtccagggctggcgagaatgtggcagaaggtgatgtcacataccctgcaagtgggaatctaaacagattcagggttttggtttttttttaatcgcaattaggtggcctgttaaattttttttcttgagacagagttttgctcttgttgcccaggctggagtgcaatggctcgatcttggctcaccgcaacctcgacctcccaggtacaagcgattctcctgtctcagcctcccaagtagctgggagtacaggtatttgccactaagcccagctaattgttttttatttagtagaaacggggtttcaccatgttagtcaggctggtcgggaactcctgacctcaggagatctacccgccttggcctcccaaagtgctgggattacaggcgtgtgccactgtgcccagccacttttttttagacagagtcttggtctgttgcccaggctagagttcagtggcgccatctcagctcactgcaacctccgcctcccagattcaagcgattctcctgcctcgacctcccagtagctgggattacaggtttccagcaaatccctctgagccgcccccgggggctcgcctcaggagcaaggaagcaaggggtgggaggaggaggtctaagtcccaggcccaattaagagatcagatggtgtaggatttgggagcttttaaggtgaagaggcccgggctgatcccactggccggtataaagcaccgtgaccctcaggtgacgcaccagggccggctgccgtcggggacagggctttccatagcc

SEQ ID NO: 3 - DNA, 529 bp, Artificial Sequence
  500 bp M opsin fragment, with M8 mutation
acaggtatttgccactaagcccagctaattgttttttatttagtagaaacggggtttcaccatgttagtcaggctggtcgggaactcctgacctcaggagatctacccgccttggcctcccaaagtgctgggattacaggcgtgtgccactgtgcccagccacttttttttagacagagtcttggtctgttgcccaggctagagttcagtggcgccatctcagctcactgcaacctccgcctcccagattcaagcgattctcctgcctcgacctcccagtagctgggattacaggtttccagcaaatccctctgagccgcccccgggggctcgcctcaggagcaaggaagcaaggggtgggaggaggaggtctaagtcccaggcccaattaagagatcagatggtgtaggatttgggagcttttaaggtgaagaggcccgggctgatcccactggccggtataaagcaccgtgaccctcaggtgacgcaccatctagagctgccgtcggggacagggctttccatagcc

SEQ ID NO: 4 - DNA, 1782 bp, Artificial Sequence
  variant of hG1.7 construct, 1.2 kb M/L opsin LCR fragment, 500 bp M opsin fragment, with M8 mutation
taggaatagaagggtgggtgcaggaggctgaggggtggggaaagggcatgggtgtttcatgaggacagagcttccgtttcatgcaatgaaaagagtttggagacggatggtggtgactggactatacacttacacacggtagcgatggtacactttgtattatgtatattttaccacgatctttttaaagtgtcaaaggcaaatggccaaatggttccttgtcctatagctgtagcagccatcggctgttagtgacaaagcccctgagtcaagatgacagcagcccccataactcctaatcggctctcccgcgtggagtcatttaggagtagtcgcattagagacaagtccaacatctaatcttccaccctggccagggccccagctggcagcgagggtgggagactccgggcagagcagagggcgctgacattggggcccggcctggcttgggtccctctggcctttccccaggggccctctttccttggggctttcttgggccgccactgctcccgctcctctccccccatcccaccccctcaccccctcgttcttcatatccttctctagtgctccctccactttcatccacccttctgcaagagtgtgggaccacaaatgagttttcacctggcctggggacacacgtgcccccacaggtgctgagtgactttctaggacagtaatctgctttaggctaaaatgggacttgatcttctgttagccctaatcatcaattagcagagccggtgaaggtgcagaacctaccgcctttccaggcctcctcccacctctgccacctccactctccttcctgggatgtgggggctggcacacgtgtggcccagggcattggtgggattgcactgagctgggtcattagcgtaatcctggacaagggcagacagggcgagcggagggccagctccggggctcaggcaaggctgggggcttcccccagacaccccactcctcctctgctggacccccacttcatagggcacttcgtgttctcaaagggcttccaaatagcatggtggccttggatgcccagggaagcctcagagttgcttatctccctctagacagaaggggaatctcggtcaagagggagaggtcgccctgttcaaggccacccagccagctcatggcggtaatgggacaaggctggccagccatcccaccctcagaagggacccggtggggcaggtgatctcagaggaggctcacttctgggtctcacattcttgacaggtatttgccactaagcccagctaattgttttttatttagtagaaacggggtttcaccatgttagtcaggctggtcgggaactcctgacctcaggagatctacccgccttggcctcccaaagtgctgggattacaggcgtgtgccactgtgcccagccacttttttttagacagagtcttggtctgttgcccaggctagagttcagtggcgccatctcagctcactgcaacctccgcctcccagattcaagcgattctcctgcctcgacctcccagtagctgggattacaggtttccagcaaatccctctgagccgcccccgggggctcgcctcaggagcaaggaagcaaggggtgggaggaggaggtctaagtcccaggcccaattaagagatcagatggtgtaggatttgggagcttttaaggtgaagaggcccgggctgatcccactggccggtataaagcaccgtgaccctcaggtgacgcaccatctagagctgccgtcggggacagggctttccatagcc

SEQ ID NO: 5 - DNA, 247 bp, Artificial Sequence
  200 bp M opsin fragment, with M8 mutation
gatcgattacaggtttccagcaaatccctctgagccgcccccgggggctcgcctcaggagcaaggaagcaaggggtgggaggaggaggtctaagtcccaggcccaattaagagatcagatggtgtaggatttgggagcttttaaggtgaagaggcccgggctgatcccactggccggtataaagcaccgtgaccctcaggtgacgcaccatctagagctgccgtcggggacagggctttccatagcc

SEQ ID NO: 6 - DNA, 1500 bp, Artificial Sequence
  hG1.4 construct: 1.2 kb M/L opsin LCR fragment, 200bp M opsin fragment, with M8 mutation
taggaatagaagggtgggtgcaggaggctgaggggtggggaaagggcatgggtgtttcatgaggacagagcttccgtttcatgcaatgaaaagagtttggagacggatggtggtgactggactatacacttacacacggtagcgatggtacactttgtattatgtatattttaccacgatctttttaaagtgtcaaaggcaaatggccaaatggttccttgtcctatagctgtagcagccatcggctgttagtgacaaagcccctgagtcaagatgacagcagcccccataactcctaatcggctctcccgcgtggagtcatttaggagtagtcgcattagagacaagtccaacatctaatcttccaccctggccagggccccagctggcagcgagggtgggagactccgggcagagcagagggcgctgacattggggcccggcctggcttgggtccctctggcctttccccaggggccctctttccttggggctttcttgggccgccactgctcccgctcctctccccccatcccaccccctcaccccctcgttcttcatatccttctctagtgctccctccactttcatccacccttctgcaagagtgtgggaccacaaatgagttttcacctggcctggggacacacgtgcccccacaggtgctgagtgactttctaggacagtaatctgctttaggctaaaatgggacttgatcttctgttagccctaatcatcaattagcagagccggtgaaggtgcagaacctaccgcctttccaggcctcctcccacctctgccacctccactctccttcctgggatgtgggggctggcacacgtgtggcccagggcattggtgggattgcactgagctgggtcattagcgtaatcctggacaagggcagacagggcgagcggagggccagctccggggctcaggcaaggctgggggcttcccccagacaccccactcctcctctgctggacccccacttcatagggcacttcgtgttctcaaagggcttccaaatagcatggtggccttggatgcccagggaagcctcagagttgcttatctccctctagacagaaggggaatctcggtcaagagggagaggtcgccctgttcaaggccacccagccagctcatggcggtaatgggacaaggctggccagccatcccaccctcagaagggacccggtggggcaggtgatctcagaggaggctcacttctgggtctcacattcttggatcgattacaggtttccagcaaatccctctgagccgcccccgggggctcgcctcaggagcaaggaagcaaggggtgggaggaggaggtctaagtcccaggcccaattaagagatcagatggtgtaggatttgggagcttttaaggtgaagaggcccgggctgatcccactggccggtataaagcaccgtgaccctcaggtgacgcaccatctagagctgccgtcggggacagggctttccatagcc

SEQ ID NO: 7 - DNA, 2085 bp, Artificial Sequence
  non-codon optimised CNGA3 cDNA
atggccaagatcaacacccaatactcccacccctccaggacccacctcaaggtaaagacctcagaccgagatctcaatcgcgctgaaaatggcctcagcagagcccactcgtcaagtgaggagacatcgtcagtgctgcagccggggatcgccatggagaccagaggactggctgactccgggcagggctccttcaccggccaggggatcgccaggctgtcgcgcctcatcttcttgctgcgcaggtgggctgccaggcatgtgcaccaccaggaccagggaccggactcttttcctgatcgtttccgtggagccgagcttaaggaggtgtccagccaagaaagcaatgcccaggcaaatgtgggcagccaggagccagcagacagagggagaagcgcctggcccctggccaaatgcaacactaacaccagcaacaacacggaggaggagaagaagacgaaaaagaaggatgcgatcgtggtggacccgtccagcaacctgtactaccgctggctgaccgccatcgccctgcctgtcttctataactggtatctgcttatttgcagggcctgtttcgatgagctgcagtccgagtacctgatgctgtggctggtcctggactactcggcagatgtcctgtatgtcttggatgtgcttgtacgagctcggacaggttttctcgagcaaggcttaatggtcagtgataccaacaggctgtggcagcattacaagacgaccacgcagttcaagctggatgtgttgtccctggtccccaccgacctggcttacttaaaggtgggcacaaactacccagaagtgaggttcaaccgcctactgaagttttcccggctctttgaattctttgaccgcacagagacaaggaccaactaccccaatatgttcaggattgggaacttggtcttgtacattctcatcatcatccactggaatgcctgcatctactttgccatttccaagttcattggttttgggacagactcctgggtctacccaaacatctcaatcccagagcatgggcgcctctccaggaagtacatttacagtctctactggtccaccttgacccttaccaccattggtgagaccccaccccccgtgaaagatgaggagtatctctttgtggtcgtagacttcttggtgggtgttctgatttttgccaccattgtgggcaatgtgggctccatgatctcgaatatgaatgcctcacgggcagagttccaggccaagattgattccatcaagcagtacatgcagttccgcaaggtcaccaaggacttggagacgcgggttatccggtggtttgactacctgtgggccaacaagaagacggtggatgagaaggaggtgctcaagagcctcccagacaagctgaaggctgagatcgccatcaacgtgcacctggacacgctgaagaaggttcgcatcttccaggactgtgaggcagggctgctggtggagctggtgctgaagctgcgacccactgtgttcagccctggggattatatctgcaagaagggagatattgggaaggagatgtacatcatcaacgagggcaagctggccgtggtggctgatgatggggtcacccagttcgtggtcctcagcgatggcagctacttcggggagatcagcattctgaacatcaaggggagcaagtcggggaaccgcaggacggccaacatccgcagcattggctactcagacctgttctgcctctcaaaggacgatctcatggaggccctcaccgagtaccccgaagccaagaaggccctggaggagaaaggacggcagatcctgatgaaagacaacctgatcgatgaggagctggccagggcgggcgcggaccccaaggaccttgaggagaaagtggagcagctggggtcctccctggacaccctgcagaccaggtttgcacgcctcctggctgagtacaacgccacccagatgaagatgaagcagcgtctcagccaactggaaagccaggtgaagggtggtggggacaagcccctggctgatggggaagttcccggggatgctacaaaaacagaggacaaacaacagtga

SEQ ID NO: 8 - DNA, 2085 bp, Artificial Sequence
  codon-optimised CNGA3 cDNA
atggcaaaaatcaatacccagtacagccacccctcacgaactcacctgaaagtcaaaacaagcgatagagacctgaacagagccgagaacggcctgtccagggcccacagctcctctgaggaaactagttcagtgctgcagcctggaatcgctatggagaccagagggctggctgactctggccaaggaagtttcacagggcagggcatcgccaggctgtctagactgatttttctgctgaggagatgggccgctaggcatgtgcaccatcaggaccagggacccgatagtttccctgacaggttcaggggggccgaactgaaggaggtcagctcccaggaatctaacgcacaggccaatgtgggcagtcaggagcccgctgatagaggacggtccgcatggcctctggccaagtgcaacactaatacctctaacaatacagaggaagagaagaaaactaagaaaaaggatgccatcgtggtcgacccttctagtaacctgtactataggtggctgacagctatcgcactgccagtgttctacaattggtatctgctgatttgcagagcttgttttgacgaactgcagagtgagtatctgatgctgtggctggtgctggattactcagcagacgtgctgtatgtgctggatgtcctggtgcgcgcacgaactgggttcctggagcagggcctgatggtgagcgacaccaacagactgtggcagcactacaaaaccacaactcagtttaagctggatgtcctgtccctggtgccaaccgacctggcctacctgaaagtcggcacaaactatcccgaggtgcggttcaatcgcctgctgaagttctctcggctgtttgagttcttcgataggacagagactagaaccaactacccaaatatgttccgcatcggcaacctggtgctgtatattctgatcattatccactggaatgcttgtatctactttgcaatcagcaagttcattggatttgggaccgacagctgggtgtatccaaacatttccatccccgaacatggacgactgagcaggaagtacatctattcactgtactggagcacactgactctgaccacaattggggagaccccccctccagtgaaggatgaagagtacctgttcgtggtcgtggactttctggtcggcgtgctgatcttcgcaacaattgtcggcaatgtgggaagtatgatctcaaacatgaatgcctcacgagctgagttccaggctaaaattgacagcatcaagcagtatatgcagtttagaaaagtcactaaggatctggagaccagagtgatccggtggtttgactacctgtgggccaacaaaaagacagtcgatgaaaaagaggtgctgaagagcctgcccgacaaactgaaggcagagattgccatcaatgtccatctggatactctgaaaaaggtgcggatcttccaggactgcgaagcaggactgctggtcgagctggtgctgaagctgcgccctaccgtgtttagcccaggcgattatatctgtaaaaagggggacattggcaaagaaatgtacattatcaacgaggggaagctggctgtcgtggcagacgatggcgtgacccagttcgtcgtgctgagcgatggcagctattttggggaaatttccatcctgaatatcaaaggctccaagtctggaaaccggcgcacagctaatattcggtccatcggatattctgacctgttctgcctgtctaaggacgatctgatggaggcactgactgaataccccgaggccaaaaaggctctggaagagaaaggccggcagatcctgatgaaggataacctgattgacgaagagctggcacgagctggagcagaccctaaagatctggaagagaaggtggagcagctgggatcaagcctggataccctgcagacacgcttcgctcgactgctggcagaatacaatgccacccagatgaaaatgaagcagcgcctgagtcagctggagtcacaggtgaaaggcggaggggacaagcccctggcagatggcgaagtccctggcgacgctacaaaaacagaagataaacagcagtaa

SEQ ID NO: 9 - DNA, 2577 bp, Artificial Sequence
  PDE6C cDNA, NM_006204.3
atgggtgagatcaaccaagttgccgtggagaaatacctggaggagaaccctcagtttgccaaggagtactttgacaggaagttgcgggtggaggtgctgggagaaatcttcaagaacagccaggtgccagtccagtccagcatgtccttctctgagctgacccaggtggaggagtcagccctgtgcttggagctgctgtggaccgtgcaggaggaggggggcaccccagagcagggggttcacagggccctgcagaggctggcccacctgctccaggctgaccgctgcagcatgttcctgtgccggtcccggaacggcatacctgaggtggcctctaggttgctggatgtcacccccacctccaagtttgaggacaacctggtgggccctgacaaagaagttgtgtttccattggacattgggatagtgggttgggctgctcacacgaagaaaactcataatgtcccagatgtgaaaaagaacagccatttttctgacttcatggacaagcaaactgggtatgtcactaagaacctgctggcaaccccgatcgtggtgggcaaggaggttcttgctgtgatcatggcagttaacaaagtaaatgcatctgaattttccaaacaggatgaagaggtcttttccaaatacctcaactttgtgtctatcatcctaaggcttcatcacaccagctacatgtacaatattgaatcccgaagaagccagatccttatgtggtcagccaataaagtatttgaagaactcacagatgttgagcgacagtttcacaaagcgctctacacggttagatcatatctgaactgtgaacgatactccattggactgctggacatgaccaaggagaaggaattctacgatgaatggccaatcaagcttggagaagtagagccttataaaggtccaaagacacctgatggcagggaagtcaacttttataaaatcattgattacattttacatggaaaagaagagatcaaagtgattccgacgcctcctgcagaccactggacactcattagtgggttgccaacatatgttgctgaaaatggatttatctgtaacatgatgaatgcccctgcggatgaatacttcacatttcagaaaggacctgtagacgaaactggttgggtcattaagaatgttttgtccctgcctattgtcaacaagaaagaagatattgtgggagtggctacattttacaacaggaaggatggaaaacctttcgatgagcatgatgaatacattaccgagactctcacacaatttcttggatggtctcttttaaatactgacacctacgataagatgaataagctagaaaacagaaaggacattgctcaggaaatgctcatgaaccaaaccaaagccactcctgaagaaattaagtccattttgaaatttcaagagaagttaaatgttgatgtaattgacgactgtgaagaaaaacaacttgttgcaattttgaaagaggacttgccagacccacgctcagcagaactgtacgaattccgcttcagtgacttcccccttacagagcacggattgattaaatgtggaatacgactgttttttgaaataaatgtggtggagaaattcaaagtacctgtagaggttcttaccagatggatgtacactgtgaggaaagggtaccgagctgtcacttaccacaattggcggcatgggttcaacgtggggcagaccatgtttactttgctgatgacaggaagattaaagaagtactacacagatctcgaagcctttgccatgcttgctgctgctttctgccatgatattgaccacagaggcaccaataatttgtaccagatgaaatccacgtctccattagcaagacttcatggttcttctattttggagaggcaccacctggagtacagtaagactctgttgcaggatgagagtttaaacatcttccagaacctaaataagcggcagtttgaaacagttattcatttgttcgaggtcgcaataatagcaactgacctggctttatatttcaagaagaggaccatgtttcaaaaaattgttgatgcctgtgaacaaatgcaaacggaagaagaagccatcaaatatgtaactgttgatccaaccaagaaagagattatcatggcaatgatgatgacggcatgtgacttgtctgctattaccaagccctgggaggtgcaaagtcaggtagcacttatggttgcaaatgaattttgggaacaaggagatctggagagaacagtgttgcagcaacaacccattcctatgatggacagaaacaaaagagatgaattacctaaacttcaagttggatttattgattttgtttgtacttttgtatataaggagttctcacggtttcacaaagaaatcacacctatgctgagtggtcttcagaataacagagtagaatggaaatcactagctgatgagtatgatgcaaagatgaaggtcattgaagaggaggcaaaaaagcaagaaggaggagccgaaaaagctgctgaagattcaggaggtggtgatgacaaaaagtccaaaacatgtttaatgttgtaa

SEQ ID NO: 10 - DNA, 252 bp, Artificial Sequence
  PDE6H cDNA, NM_006205.2
atgagtgacaacactactctgcctgctccagcttcaaaccagggtcctaccaccccacgcaaaggccctcccaagttcaagcagaggcagactcgccaattcaagagtaaacctccaaagaaaggtgtgaaaggatttggagatgacattccaggaatggaggggctaggaacagatatcacagtgatttgtccatgggaggcattcagccacctggaattgcatgagctcgctcagtttgggattatctga

SEQ ID NO: 11 - DNA, 1065 bp, Artificial Sequence
  GNAT2 cDNA, NM_005272.3
atgggaagtggagccagtgctgaggacaaagaactggccaagaggtccaaggagctagaaaagaagctgcaggaggatgctgataaggaagccaagactgtcaagctgctactgctgggtgctggggagtcaggaaagagcaccatcgtcaaacagatgaagatcattcaccaggatggctattcaccagaagaatgcctggagttcaaggctatcatctatggaaatgtgctgcagtccatcctggctatcatccgggccatgaccacactgggcatcgattatgctgaaccaagctgtgcggatgacgggcgacagctcaacaacctggctgactccattgaggagggaaccatgcctcctgagctcgtggaggtcattaggaggttgtggaaggatggtggggtgcaagcctgcttcgagagagctgcagaataccagcttaatgactccgcatcttactacctgaaccaattagaacgaattacagaccctgagtacctccctagtgagcaagatgtgctccgatccagagtcaaaaccacgggcatcattgaaaccaagttttccgtcaaagacttgaatttcaggatgtttgatgtgggagggcagagatccgagagaaagaagtggatccactgcttcgagggagtcacctgcatcattttctgtgcagccctcagtgcctatgatatggtgctggtggaagatgacgaagtgaatcgtatgcatgagtctttgcatctgttcaacagcatatgtaaccacaaattctttgcggctacttccattgtcctctttctcaacaagaaggacctctttgaggaaaaaatcaagaaagtccatctcagcatttgttttccagagtatgatggtaacaactcctatgatgatgcggggaattacataaagagccagttccttgacctcaatatgcgaaaagatgtcaaagaaatctacagtcacatgacctgtgctacagatacacagaatgtcaaatttgtgtttgatgcagttacagatattatcatcaaagaaaacctcaaggactgcggcctcttctaa

SEQ ID NO: 12 - DNA, 1638 bp, Artificial Sequence
  KCNV2 cDNA, NM_133497.3
atgctcaaacagagtgagaggagacggtcctggagctacaggccctggaacacgacggagaatgagggcagccaacaccgcaggagcatttgctccctgggtgcccgttccggctcccaggccagcatccacggctggacagagggcaactataactactacatcgaggaagacgaagacggcgaggaggaggaccagtggaaggacgacctggcagaagaggaccagcaggcaggggaggtcaccaccgccaagcccgagggccccagcgaccctccggccctgctgtccacgctgaatgtgaacgtgggtggccacagctaccagctggactactgcgagctggccggcttccccaagacgcgcctaggtcgcctggccacctccaccagccgcagccgccagctaagcctgtgcgacgactacgaggagcagacagacgaatacttcttcgaccgcgacccggccgtcttccagctggtctacaatttctacctgtccggggtgctgctggtgctcgacgggctgtgtccgcgccgcttcctggaggagctgggctactggggcgtgcggctcaagtacacgccacgctgctgccgcatctgcttcgaggagcggcgcgacgagctgagcgaacggctcaagatccagcacgagctgcgcgcgcaggcgcaggtcgaggaggcggaggaactcttccgcgacatgcgcttctacggcccgcagcggcgccgcctctggaacctcatggagaagccattctcctcggtggccgccaaggccatcggggtggcctccagcaccttcgtgctcgtctccgtggtggcgctggcgctcaacaccgtggaggagatgcagcagcactcggggcagggcgagggcggcccagacctgcggcccatcctggagcacgtggagatgctgtgcatgggcttcttcacgctcgagtacctgctgcgcctagcctccacgcccgacctgaggcgcttcgcgcgcagcgccctcaacctggtggacctggtggccatcctgccgctctaccttcagctgctgctcgagtgcttcacgggcgagggccaccaacgcggccagacggtgggcagcgtgggtaaggtgggtcaggtgttgcgcgtcatgcgcctcatgcgcatcttccgcatcctcaagctggcgcgccactccaccggactgcgtgccttcggcttcacgctgcgccagtgctaccagcaggtgggctgcctgctgctcttcatcgccatgggcatcttcactttctctgcggctgtctactctgtggagcacgatgtgcccagcaccaacttcactaccatcccccactcctggtggtgggccgcggtgagcatctccaccgtgggctacggagacatgtacccagagacccacctgggcaggttttttgccttcctctgcattgcttttgggatcattctcaacgggatgcccatttccatcctctacaacaagttttctgattactacagcaagctgaaggcttatgagtataccaccatacgcagggagaggggagaggtgaacttcatgcagagagccagaaagaagatagctgagtgtttgcttggaagcaacccacagctcaccccaagacaagagaattag

SEQ ID NO: 13 - DNA, 3414 bp, Artificial Sequence
  CACNA2D4 cDNA, NM_172364.4
atggtctgtggctgctctgccctccttcccctccccaaccccaggcccaccatgcctgcaactcccaacttcctcgcaaaccccagctccagcagccgctggattcccctccagccaatgcccgtggcctgggcctttgtgcagaagacctcggccctcctgtggctgctgcttctaggcacctccctgtcccctgcgtggggacaggccaagattcctctggaaacagtgaagctatgggctgacaccttcggcggggacctgtataacactgtgaccaaatactcaggctctctcttgctgcagaagaagtacaaggatgtggagtccagtctgaagatcgaggaggtggatggcttggagctggtgaggaagttctcagaggacatggagaacatgctgcggaggaaagtcgaggcggtccagaatctggtggaagctgccgaggaggccgacctgaaccacgaattcaatgaatccctggtgttcgactattacaactcggtcctgatcaacgagagggacgagaagggcaacttcgtggagctgggcgccgagttcctcctggagtccaatgctcacttcagcaacctgccggtgaacacctccatcagcagcgtgcagctgcccaccaacgtgtacaacaaagacccagatattttaaatggagtctacatgtctgaagccttgaatgctgtcttcgtggagaacttccagagagacccaacgttgacctggcaatattttggcagtgcaactggattcttcaggatctatccaggtataaaatggacacctgatgagaatggagtcattacttttgactgccgaaaccgcggctggtacattcaagctgctacttctcccaaggacatagtgattttggtggacgtgagcggcagtatgaaggggctgaggatgactattgccaagcacaccatcaccaccatcttggacaccctgggggagaatgacttcattaatatcatagcgtacaatgactacgtccattacatcgagccttgttttaaagggatcctcgtccaggcggaccgagacaatcgagagcatttcaaactgctggtggaggagttgatggtcaaaggtgtgggggtcgtggaccaagccctgagagaagccttccagatcctgaagcagttccaagaggccaagcaaggaagcctctgcaaccaggccatcatgctcatcagcgacggcgccgtggaggactacgagccggtgtttgagaagtataactggccagactgtaaggtccgagttttcacttacctcattgggagagaagtgtcttttgctgaccgcatgaagtggattgcatgcaacaacaaaggctactacacgcagatctcaacgctggcggacacccaggagaacgtgatggaatacctgcacgtgctcagccgccccatggtcatcaaccacgaccacgacatcatctggacagaggcctacatggacagcaagctcctcagctcgcaggctcagagcctgacactgctcaccactgtggccatgccagtcttcagcaagaagaacgaaacgcgatcccatggcattctcctgggtgtggtgggctcagatgtggccctgagagagctgatgaagctggcgccccggtacaagcttggagtgcacggatacgcctttctgaacaccaacaatggctacatcctctcccatcccgacctccggcccctgtacagagaggggaagaaactaaaacccaaacctaactacaacagtgtggatctctccgaagtggagtgggaagaccaggctgaatctctgagaacagccatgatcaatagggaaacaggtactctctcgatggatgtgaaggttccgatggataaagggaagcgagttcttttcctgaccaatgactacttcttcacggacatcagcgacacccctttcagtttgggggtggtgctgtcccggggccacggagaatacatccttctggggaacacgtctgtggaagaaggcctgcatgacttgcttcacccagacctggccctggccggtgactggatctactgcatcacagatattgacccagaccaccggaagctcagccagctagaggccatgatccgcttcctcaccaggaaggacccagacctggagtgtgacgaggagctggtccgggaggtgctgtttgacgcggtggtgacagcccccatggaagcctactggacagcgctggccctcaacatgtccgaggagtctgaacacgtggtggacatggccttcctgggcacccgggctggcctcctgagaagcagcttgttcgtgggctccgagaaggtctccgacaggaagttcctgacacctgaggacgaggccagcgtgttcaccctggaccgcttcccgctgtggtaccgccaggcctcagagcatcctgctggcagcttcgtcttcaacctccgctgggcagaaggaccagaaagtgcgggtgaacccatggtggtgacggcaagcacagctgtggcggtgaccgtggacaagaggacagccattgctgcagccgcgggcgtccaaatgaagctggaattcctccagcgcaaattctgggcggcaacgcggcagtgcagcactgtggatgggccgtgcacacagagctgcgaggacagtgatctggactgcttcgtcatcgacaacaacgggttcattctgatctccaagaggtcccgagagacgggaagatttctgggggaggtggatggtgctgtcctgacccagctgctcagcatgggggtgttcagccaagtgactatgtatgactatcaggccatgtgcaaaccctcgagtcaccaccacagtgcagcccagcccctggtcagcccaatttctgccttcttgacggcgaccaggtggctgctgcaggagctggtgctgttcctgctggagtggagtgtctggggctcctggtacgacagaggggccgaggccaaaagtgtcttccatcactcccacaaacacaagaagcaggacccgctgcagccctgcgacacggagtaccccgtgttcgtgtaccagccggccatccgggaggccaacgggatcgtggagtgcgggccctgccagaaggtatttgtggtgcagcagattcccaacagtaacctcctcctcctggtgacagaccccacctgtgactgcagcatcttcccaccagtgctgcaggaggcgacagaagtcaaatataatgcctctgtcaaatgtgaccggatgcgctcccagaagctccgccggcgaccagactcctgccacgccttccatccagaggagaatgcccaggactgcggcggcgcctcggacacctcagcctcgccgcccctactcctgctgcctgtgtgtgcctgggggctactgccccaactcctgcggtga

SEQ ID NO: 14 - DNA, 2430 bp, Artificial Sequence
  CNGB3 cDNA, NM_019098.4
atgtttaaatcgctgacaaaagtcaacaaggtgaagcctataggagagaacaatgagaatgaacaaagttctcgtcggaatgaagaaggctctcacccaagtaatcagtctcagcaaaccacagcacaggaagaaaacaaaggtgaagagaaatctctcaaaaccaagtcaactccagtcacgtctgaagagccacacaccaacatacaagacaaactctccaagaaaaattcctctggagatctgaccacaaaccctgaccctcaaaatgcagcagaaccaactggaacagtgccagagcagaaggaaatggaccccgggaaagaaggtccaaacagcccacaaaacaaaccgcctgcagctcctgttataaatgagtatgccgatgcccagctacacaacctggtgaaaagaatgcgtcaaagaacagccctctacaagaaaaagttggtagagggagatctctcctcacccgaagccagcccacaaactgcaaagcccacggctgtaccaccagtaaaagaaagcgatgataagccaacagaacattactacaggctgttgtggttcaaagtcaaaaagatgcctttaacagagtacttaaagcgaattaaacttccaaacagcatagattcatacacagatcgactctatctcctgtggctcttgcttgtcactcttgcctataactggaactgctggtttataccactgcgcctcgtcttcccatatcaaaccgcagacaacatacactactggcttattgcggacatcatatgtgatatcatctacctttatgatatgctatttatccagcccagactccagtttgtaagaggaggagacataatagtggattcaaatgagctaaggaaacactacaggacttctccaaaatttcagttggatgtcgcatcaataataccatttgatatttgctacctcttctttgggtttaatccaatgtttagagcaaataggatgttaaagtacacttcattttttgaatttaatcatcacctagagtctataatggacaaagcatatatctacagagttattcgaacaactggatacttgctgtttattctgcacattaatgcctgtgtttattactgggcttcaaactatgaaggaattggcactactagatgggtgtatgatggggaaggaaacgagtatctgagatgttattattgggcagttcgaactttaattaccattggtggcctaccagaaccacaaactttatttgaaattgtttttcaactcttgaattttttttctggagtttttgtgttctccagtttaattggtcagatgagagatgtgattggagcagctacagccaatcagaactacttccgcgcctgcatggatgacaccattgcctacatgaacaattactccattcctaaacttgtgcaaaagcgagttcggacttggtatgaatatacatgggactctcaaagaatgctagatgagtctgatttgcttaagaccctaccaactacggtccagttagccctcgccattgatgtgaacttcagcatcatcagcaaagtcgacttgttcaagggttgtgatacacagatgatttatgacatgttgctaagattgaaatccgttctctatttgcctggtgactttgtctgcaaaaagggagaaattggcaaggaaatgtatatcatcaagcatggagaagtccaagttcttggaggccctgatggtactaaagttctggttactctgaaagctgggtcggtgtttggagaaatcagccttctagcagcaggaggaggaaaccgtcgaactgccaatgtggtggcccacgggtttgccaatcttttaactctagacaaaaagaccctccaagaaattctagtgcattatccagattctgaaaggatcctcatgaagaaagccagagtgcttttaaagcagaaggctaagaccgcagaagcaacccctccaagaaaagatcttgccctcctcttcccaccgaaagaagagacacccaaactgtttaaaactctcctaggaggcacaggaaaagcaagtcttgcaagactactcaaattgaagcgagagcaagcagctcagaagaaagaaaattctgaaggaggagaggaagaaggaaaagaaaatgaagataaacaaaaagaaaatgaagataaacaaaaagaaaatgaagataaaggaaaagaaaatgaagataaagataaaggaagagagccagaagagaagccactggacagacctgaatgtacagcaagtcctattgcagtggaggaagaaccccactcagttagaaggacagttttacccagagggacttctcgtcaatcactcattatcagcatggctccttctgctgagggcggagaagaggttcttactattgaagtcaaagaaaaggctaagcaataa

SEQ ID NO: 15 - DNA, 1786 bp, Artificial Sequence
  hG1.7 construct , 1.2 kb M/L opsin LCR fragment, 500 bp M opsin fragment, with M8 mutation
taggaatagaagggtgggtgcaggaggctgaggggtggggaaagggcatgggtgtttcatgaggacagagcttccgtttcatgcaatgaaaagagtttggagacggatggtggtgactggactatacacttacacacggtagcgatggtacactttgtattatgtatattttaccacgatctttttaaagtgtcaaaggcaaatggccaaatggttccttgtcctatagctgtagcagccatcggctgttagtgacaaagcccctgagtcaagatgacagcagcccccataactcctaatcggctctcccgcgtggagtcatttaggagtagtcgcattagagacaagtccaacatctaatcttccaccctggccagggccccagctggcagcgagggtgggagactccgggcagagcagagggcgctgacattggggcccggcctggcttgggtccctctggcctttccccaggggccctctttccttggggctttcttgggccgccactgctcccgctcctctccccccatcccaccccctcaccccctcgttcttcatatccttctctagtgctccctccactttcatccacccttctgcaagagtgtgggaccacaaatgagttttcacctggcctggggacacacgtgcccccacaggtgctgagtgactttctaggacagtaatctgctttaggctaaaatgggacttgatcttctgttagccctaatcatcaattagcagagccggtgaaggtgcagaacctaccgcctttccaggcctcctcccacctctgccacctccactctccttcctgggatgtgggggctggcacacgtgtggcccagggcattggtgggattgcactgagctgggtcattagcgtaatcctggacaagggcagacagggcgagcggagggccagctccggggctcaggcaaggctgggggcttcccccagacaccccactcctcctctgctggacccccacttcatagggcacttcgtgttctcaaagggcttccaaatagcatggtggccttggatgcccagggaagcctcagagttgcttatctccctctagacagaaggggaatctcggtcaagagggagaggtcgccctgttcaaggccacccagccagctcatggcggtaatgggacaaggctggccagccatcccaccctcagaagggacccggtggggcaggtgatctcagaggaggctcacttctgggtctcacattcttggatcacaggtatttgccactaagcccagctaattgttttttatttagtagaaacggggtttcaccatgttagtcaggctggtcgggaactcctgacctcaggagatctacccgccttggcctcccaaagtgctgggattacaggcgtgtgccactgtgcccagccacttttttttagacagagtcttggtctgttgcccaggctagagttcagtggcgccatctcagctcactgcaacctccgcctcccagattcaagcgattctcctgcctcgacctcccagtagctgggattacaggtttccagcaaatccctctgagccgcccccgggggctcgcctcaggagcaaggaagcaaggggtgggaggaggaggtctaagtcccaggcccaattaagagatcagatggtgtaggatttgggagcttttaaggtgaagaggcccgggctgatcccactggccggtataaagcaccgtgaccctcaggtgacgcaccatctagagctgccgtcggggacagggctttccatagcc

SEQ ID NO: 16 - DNA, 6 bp, Artificial Sequence
  M8 mutation
tctaga

SEQ ID NO: 17 - DNA, 1970 bp, Artificial Sequence
  2.0 kb M opsin promoter fragment with M8 mutation
taaaaagcaagtcttgccagggcagtggtgtgcacctgtggtcccagctactcaggatgctgaggcaggaggattacttgtgcccagcaagtagaggctgcagtgacctgtgactgtgctactgccctccaacctgggtgacagagtgagaccttgtctcaaaaaaaaaagagcggggggggggggccgggccgggcgtggtggctcacagctgtaatcccagcactttgggaagccaaggcgggtggatcacttgaggtcaggagtttgagaccatcatggtcaacactgcgaaacactgtccctactaaaaatacaaaaattagccgggcatggtggcacacacctgtaatcccagctactggggaggctgaggcaggagaattgcttgagccggggagacggaggttgcagtgagccgagactgcgccactgcactccagcctgactgacaagagtgagattgtctcaaaaaaaaaaaaaaagtaatcactagaaaagaagctacatatgtacataacatccaaataaccaagaggagaaaaaaatgggacttgattaatcaaaacaaaaacaaaaaagaaagaaagaaagggggagaaaataaaacaagggctgggtgtgctggctcatgcctgtaatcccagcactttggaagccaaggtgggtggatctcttgagctcaggaggtcaagaccagcctgggcaacatggcgaaaccccgtctctattaaaaaaaaaattaatacaacaattatcctggagtggtggtgcacacctgtagtcccagctacccaggacgctgagacgggaggatcgcttgatcccggggatgtcgaggctgccgtgatcgcaccactgccctccagccagggtggcagactgagaccccatctcaaaaaataaataaataaaagcaaacaagaaaaaaaaaggcttgaaacatatctgatagataaagggctaatcaacacaatatataaagaactgcaaatcagtaaactaagagcaaataacccaatataaagacattaaagggtagccacggacatctcagacgacgaaaaacaaaagacagtaaacgtataataaaacatgtaattgcaaggtgatccgggaatagtaagcgaaaagcaacaattaaatactattttctcatccaccagaacgccaaaaattaaaaagcctaacaatgtccagggctggcgagaatgtggcagaaggtgatgtcacataccctgcaagtgggaatctaaacagattcagggttttggtttttttttaatcgcaattaggtggcctgttaaattttttttcttgagacagagttttgctcttgttgcccaggctggagtgcaatggctcgatcttggctcaccgcaacctcgacctcccaggtacaagcgattctcctgtctcagcctcccaagtagctgggagtacaggtatttgccactaagcccagctaattgttttttatttagtagaaacggggtttcaccatgttagtcaggctggtcgggaactcctgacctcaggagatctacccgccttggcctcccaaagtgctgggattacaggcgtgtgccactgtgcccagccacttttttttagacagagtcttggtctgttgcccaggctagagttcagtggcgccatctcagctcactgcaacctccgcctcccagattcaagcgattctcctgcctcgacctcccagtagctgggattacaggtttccagcaaatccctctgagccgcccccgggggctcgcctcaggagcaaggaagcaaggggtgggaggaggaggtctaagtcccaggcccaattaagagatcagatggtgtaggatttgggagcttttaaggtgaagaggcccgggctgatcccactggccggtataaagcaccgtgaccctcaggtgacgcaccatctagagctgccgtcggggacagggctttccatagcc